European Patent Application EP 4 245 772 A1, published September 20, 2023. Title: Anti-netrin-1 antibody to treat liver inflammation. Applicant: NETRIS PHARMA. The sequence listing filed with the application follows.

SEQUENCE LISTING (34 sequences)

SEQ ID NO: 1 - protein, 604 aa, Homo sapiens
  SIGNAL (1)..(24)
  MISC_FEATURE (339)..(381): linear epitope
MMRAVWEALAALAAVACLVGAVRGGPGLSMFAGQAAQPDPCSDENGHPRRCIPDFVNAAFGKDVRVSSTCGRPPARYCVVSERGEERLRSCHLCNASDPKKAHPPAFLTDLNNPHNLTCWQSENYLQFPHNVTLTLSLGKKFEVTYVSLQFCSPRPESMAIYKSMDYGRTWVPFQFYSTQCRKMYNRPHRAPITKQNEQEAVCTDSHTDMRPLSGGLIAFSTLDGRPSAHDFDNSPVLQDWVTATDIRVAFSRLHTFGDENEDDSELARDSYFYAVSDLQVGGRCKCNGHAARCVRDRDDSLVCDCRHNTAGPECDRCKPFHYDRPWQRATAREANECVACNCNLHARRCRFNMELYKLSGRKSGGVCLNCRHNTAGRHCHYCKEGYYRDMGKPITHRKACKACDCHPVGAAGKTCNQTTGQCPCKDGVTGITCNRCAKGYQQSRSPIAPCIKIPVAPPTTAASSVEEPEDCDSYCKASKGKLKINMKKYCKKDYAVQIHILKADKAGDWWKFTVNIISVYKQGTSRIRRGDQSLWIRSRDIACKCPKIKPLKKYLLLGNAEDSPDQSGIVADKSSLVIQWRDTWARRLRKFQQREKKGKCKKA

SEQ ID NO: 2 - DNA, 1817 bp, Homo sapiens
atgatgcgcgcagtgtgggaggcgctggcggcgctggcggcggtggcgtgcctggtgggcgcggtgcgcggcgggcccgggctcagcatgttcgcgggccaggcggcgcagcccgatccctgctcggacgagaacggccacccgcgccgctgcatcccggactttgtcaatgcggccttcggcaaggacgtgcgcgtgtccagcacctgcggccggcccccggcgcgctactgcgtggtgagcgagcgcggcgaggagcggctgcgctcgtgccacctctgcaacgcgtccgaccccaagaaggcgcacccgcccgccttcctcaccgacctcaacaacccgcacaacctgacgtgctggcagtccgagaactacctgcagttcccgcacaacgtcacgctcacactgtccctcggcaagaagttcgaagtgacctacgtgagcctgcagttctgctcgccgcggcccgagtccatggccatctacaagtccatggactacgggcgcacgtgggtgcccttccagttctactccacgcagtgccgcaagatgtacaaccggccgcaccgcgcgcccatcaccaagcagaacgagcaggaggccgtgtgcaccgactcgcacaccgacatgcgcccgctctcgggcggcctcatcgccttcagcacgctggacgggcggccctcggcgcacgacttcgacaactcgcccgtgctgcaggactgggtcacggccacagacatccgcgtggccttcagccgcctgcacacgttcggcgacgagaacgaggacgactcggagctggcgcgcgactcgtacttctacgcggtgtccgacctgcaggtgggcggccggtgcaagtgcaacggccacgcggcccgctgcgtgcgcgaccgcgacgacagcctggtgtgcgactgcaggcacaacacggccggcccggagtgcgaccgctgcaagcccttccactacgaccggccctggcagcgcgccacagcccgcgaagccaacgagtgcgtggcctgtaactgcaacctgcatgcccggcgctgccgcttcaacatggagctctacaagctttcggggcgcaagagcggaggtgtctgcctcaactgtcgccacaacaccgccggccgccactgccattactgcaaggagggctactaccgcgacatgggcaagcccatcacccaccggaaggcctgcaaagcctgtgattgccaccctgtgggtgctgctggcaaaacctgcaaccaaaccaccggccagtgtccctgcaaggacggcgtgacgggtatcacctgcaaccgctgcgccaaaggctaccagcagagccgctctcccatcgccccctgcataaagatccctgtagcgccgccgacgactgcagccagcagcgtggaggagcctgaagactgcgattcctactgcaaggcctccaaggggaagctgaagattaacatgaaaaagtactgcaagaaggactatgccgtccagatccacatcctgaaggcggacaaggcgggggactggtggaagttcacggtgaacatcatctccgtgtataagcagggcacgagccgcatccgccgcggtgaccagagcctgtggatccgctcgcgggacatcgcctgcaagtgtcccaaaatcaagcccctcaagaagtacctgctgctgggcaacgcggaggactctccggaccagagcggcatcgtggccgataaaagcagcctggtgatccagtggcgggacacgtgggcgcggcggctgcgcaagttccagcagcgtgagaagaagggcaagtgcaagaaggcctagcg

SEQ ID NO: 3 - protein, 43 aa, Homo sapiens
VACNCNLHARRCRFNMELYKLSGRKSGGVCLNCRHNTAGRHCH

SEQ ID NO: 4 - DNA, 129 bp, Homo sapiens
gtggcctgtaactgcaacctgcatgcccggcgctgccgcttcaacatggagctctacaagctttcggggcgcaagagcggaggtgtctgcctcaactgtcgccacaacaccgccggccgccactgccat

SEQ ID NO: 5 - protein, 8 aa, Mus musculus
GYTFTSYN

SEQ ID NO: 6 - protein, 8 aa, Mus musculus
IYPGNGDT

SEQ ID NO: 7 - protein, 9 aa, Mus musculus
ARGGTGFAY

SEQ ID NO: 8 - protein, 6 aa, Mus musculus
QSVSND

SEQ ID NO: 9 - protein, 9 aa, Mus musculus
QQDYSSPWT

SEQ ID NO: 10 - protein, 116 aa, Mus musculus
  MISC_FEATURE (26)..(33): CDR according to IGMT
  MISC_FEATURE (51)..(58): CDR according to IGMT
  MISC_FEATURE (97)..(105): CDR according to IGMT
QAYLQQSGAELVRPGASVKMSCKASGYTFTSYNMHWVKQTPRQGLEWIGAIYPGNGDTSYNQKFKGKATLTVDKSSSTAYMQLSSLTSEDSAVYFCARGGTGFAYWGQGTLVTVSA

SEQ ID NO: 11 - protein, 107 aa, Mus musculus
  MISC_FEATURE (27)..(32): CDR according to IGMT
  MISC_FEATURE (50)..(52): CDR according to IGMT
  MISC_FEATURE (89)..(97): CDR according to IGMT
SIVMTQTPKFLLVSAGDRVTITCKASQSVSNDVAWYQQKPGQSPKLLIYYASNRYTGVPDRFTGSGYGTDFTFTISTVQAEDLAVYFCQQDYSSPWTFGGGTKLEIK

SEQ ID NO: 12 - protein, 440 aa, Mus musculus
  MISC_FEATURE (26)..(33): CDR according to IGMT
  MISC_FEATURE (51)..(58): CDR according to IGMT
  MISC_FEATURE (97)..(105): CDR according to IGMT
QAYLQQSGAELVRPGASVKMSCKASGYTFTSYNMHWVKQTPRQGLEWIGAIYPGNGDTSYNQKFKGKATLTVDKSSSTAYMQLSSLTSEDSAVYFCARGGTGFAYWGQGTLVTVSAAKTTPPSVYPLAPGSAAQTNSMVTLGCLVKGYFPEPVTVTWNSGSLSSGVHTFPAVLESDLYTLSSSVTVPSSPRPSETVTCNVAHPASSTKVDKKIVPRDCGCKPCICTVPEVSSVFIFPPKPKDVLTITLTPKVTCVVVDISKDDPEVQFSWFVDDVEVHTAQTQPREEQFNSTFRSVSELPIMHQDWLNGKEFKCRVNSAAFPAPIEKTISKTKGRPKAPQVYTIPPPKEQMAKDKVSLTCMITDFFPEDITVEWQWNGQPAENYKNTQPIMNTNGSYFVYSKLNVQKSNWEAGNTFTCSVLHEGLHNHHTEKSLSHSPGK

SEQ ID NO: 13 - protein, 214 aa, Mus musculus
  MISC_FEATURE (27)..(32): CDR according to IGMT
  MISC_FEATURE (50)..(52): CDR according to IGMT
  MISC_FEATURE (89)..(97): CDR according to IGMT
SIVMTQTPKFLLVSAGDRVTITCKASQSVSNDVAWYQQKPGQSPKLLIYYASNRYTGVPDRFTGSGYGTDFTFTISTVQAEDLAVYFCQQDYSSPWTFGGGTKLEIKRADAAPTVSIFPPSSEQLTSGGASVVCFLNNFYPKDINVKWKIDGSERQNGVLNSWTDQDSKDSTYSMSSTLTLTKDEYERHNSYTCEATHKTSTSPIVKSFNRNEC

SEQ ID NO: 14 - protein, 101 aa, Artificial Sequence
  humanized variant
  MISC_FEATURE (27)..(32): CDR according to IGMT
  MISC_FEATURE (50)..(52): CDR according to IGMT
  MISC_FEATURE (89)..(97): CDR according to IGMT
EIVMTQSPATLSVSPGERATLSCKASQSVSNDVAWYQQKPGKAPKLLIYYASNRYTGIPPRFSGSGYGTDFTLTINNIESEDAAYYFCQQDYSSPWTFGQG

SEQ ID NO: 15 - protein, 101 aa, Artificial Sequence
  humanized variant
  MISC_FEATURE (27)..(32): CDR according to IGMT
  MISC_FEATURE (50)..(52): CDR according to IGMT
  MISC_FEATURE (89)..(97): CDR according to IGMT
DIQMTQSPSSLSASVGDRVTITCKASQSVSNDVAWFQQRPGQSPRRLIYYASNRYTGVPSRFSGSGSGTDFTFTISSLEAEDAATYYCQQDYSSPWTFGQG

SEQ ID NO: 16 - protein, 101 aa, Artificial Sequence
  humanized variant
  MISC_FEATURE (27)..(32): CDR according to IGMT
  MISC_FEATURE (50)..(52): CDR according to IGMT
  MISC_FEATURE (89)..(97): CDR according to IGMT
DIQMTQSPSSLSASVGDRVTITCKASQSVSNDVAWYQQKPGQAPRLLIYYASNRYTGIPPRFSGSGYGTDFTLTINNIESEDAAYYFCQQDYSSPWTFGQG

SEQ ID NO: 17 - protein, 101 aa, Artificial Sequence
  humanized variant
  MISC_FEATURE (27)..(32): CDR according to IGMT
  MISC_FEATURE (50)..(52): CDR according to IGMT
  MISC_FEATURE (89)..(97): CDR according to IGMT
DIQMTQSPSSLSASVGDRVTITCKASQSVSNDVAWYLQKPGQSPQLLIYYASNRYTGVPSRFSGSGSGTDFTFTISSLEAEDAATYYCQQDYSSPWTFGQG

SEQ ID NO: 18 - protein, 101 aa, Artificial Sequence
  humanized variant
  MISC_FEATURE (27)..(32): CDR according to IGMT
  MISC_FEATURE (50)..(52): CDR according to IGMT
  MISC_FEATURE (89)..(97): CDR according to IGMT
DIVMTQTPLSLPVTPGEPASISCKASQSVSNDVAWYQQKPGQAPRLLIYYASNRYTGIPPRFSGSGYGTDFTLTINNIESEDAAYYFCQQDYSSPWTFGQG

SEQ ID NO: 19 - protein, 101 aa, Artificial Sequence
  humanized variant
  MISC_FEATURE (27)..(32): CDR according to IGMT
  MISC_FEATURE (50)..(52): CDR according to IGMT
  MISC_FEATURE (89)..(97): CDR according to IGMT
EIVMTQSPATLSVSPGERATLSCRASQSVSNDVAWYQQKPGQAPRLLIYYASNRYTGIPARFSGSGSGTEFTLTISSLQSEDFAVYYCQQDYSSPWTFGQG

SEQ ID NO: 20 - protein, 109 aa, Artificial Sequence
  humanized variant
  MISC_FEATURE (26)..(33): CDR according to IGMT
  MISC_FEATURE (51)..(58): CDR according to IGMT
  MISC_FEATURE (97)..(105): CDR according to IGMT
QVQLVQSGAEVKKPGASVKVSCKASGYTFTSYNMHWVRQATGQGLEWMGAIYPGNGDTSYNQKFKGRVTITADKSTSTAYMELSSLRSEDTAVYYCARGGTGFAYWGQG

SEQ ID NO: 21 - protein, 109 aa, Artificial Sequence
  humanized variant
  MISC_FEATURE (26)..(33): CDR according to IGMT
  MISC_FEATURE (51)..(58): CDR according to IGMT
  MISC_FEATURE (97)..(105): CDR according to IGMT
QVQLQQSGPGLVKPSQTLSLTCAISGYTFTSYNMHWIRQPPGKGLEWIGAIYPGNGDTSYNQKFKGRVTITADKSTSTAYMELSSLRSEDTAVYYCARGGTGFAYWGQG

SEQ ID NO: 22 - protein, 109 aa, Artificial Sequence
  humanized variant
  MISC_FEATURE (26)..(33): CDR according to IGMT
  MISC_FEATURE (51)..(58): CDR according to IGMT
  MISC_FEATURE (97)..(105): CDR according to IGMT
QVQLQQSGPGLVKPSQTLSLTCAISGYTFTSYNMHWVRQATGQGLEWMGAIYPGNGDTSYNQKFKGRLTISKDTSKNQVVLTMTNMDPVDTATYYCARGGTGFAYWGQG

SEQ ID NO: 23 - protein, 109 aa, Artificial Sequence
  humanized variant
  MISC_FEATURE (26)..(33): CDR according to IGMT
  MISC_FEATURE (51)..(58): CDR according to IGMT
  MISC_FEATURE (97)..(105): CDR according to IGMT
EVQLVQSGAEVKKPGESLRISCKGSGYTFTSYNMHWVRQATGQGLEWMGAIYPGNGDTSYNQKFKGRFTISRDDSKNTAYLQMNSLKTEDTAVYYCARGGTGFAYWGQG

SEQ ID NO: 24 - protein, 109 aa, Artificial Sequence
  humanized variant
  MISC_FEATURE (26)..(33): CDR according to IGMT
  MISC_FEATURE (51)..(58): CDR according to IGMT
  MISC_FEATURE (97)..(105): CDR according to IGMT
QVQLQESGPGLVKPSQTLSLTCTVSGYTFTSYNMHWVRQAPGQGLEWMGAIYPGNGDTSYNQKFKGRVTISVDTSKNQFSLKLSSVTAADTAVYYCARGGTGFAYWGQG

SEQ ID NO: 25 - protein, 109 aa, Artificial Sequence; identical to SEQ ID NO: 20
  humanized variant
  MISC_FEATURE (26)..(33): CDR according to IGMT
  MISC_FEATURE (51)..(58): CDR according to IGMT
  MISC_FEATURE (97)..(105): CDR according to IGMT

SEQ ID NO: 26 - protein, 109 aa, Artificial Sequence
  humanized variant
  MISC_FEATURE (26)..(33): CDR according to IGMT
  MISC_FEATURE (51)..(58): CDR according to IGMT
  MISC_FEATURE (97)..(105): CDR according to IGMT
QVQLQQSGPGLVKPSQTLSLTCAISGYTFTSYNMHWVRQATGQGLEWMGAIYPGNGDTSYNQKFKGRVTITADKSTSTAYMELSSLRSEDTAVYYCARGGTGFAYWGQG

SEQ ID NO: 27 - protein, 108 aa, Artificial Sequence
  humanized variant
  MISC_FEATURE (26)..(33): CDR according to IGMT
  MISC_FEATURE (51)..(58): CDR according to IGMT
  MISC_FEATURE (97)..(105): CDR according to IGMT
QVQLVQSGAEVKKPGASVKVSCKASGYTFTSYNMHWVRQAPGQGLEWMGAIYPGNGDTSYAQKFKGRVTMTRDTSTSTVYMELSSLRSEDTAVYYCARGGTGFAYWGQ

SEQ ID NO: 28 - protein, 5 aa, Mus musculus
SYNMH

SEQ ID NO: 29 - protein, 17 aa, Mus musculus
AIYPGNGDTSYNQKFKG

SEQ ID NO: 30 - protein, 7 aa, Mus musculus
GGTGFAY

SEQ ID NO: 31 - protein, 11 aa, Mus musculus
KASQSVSNDVA

SEQ ID NO: 32 - protein, 7 aa, Mus musculus
YASNRYT

SEQ ID NO: 33 - protein, 22 aa, Homo sapiens
ARRCRFNMELYKLSGRKSGGVC

SEQ ID NO: 34 - DNA, 66 bp, cDNA
gcccggcgctgccgcttcaacatggagctctacaagctttcggggcgcaagagcggaggtgtctgc